European Patent Application EP 4 458 991 A1, published November 6, 2024. Title: 一种用于检测的引物探针、引物探针组及其应用. Applicant: 迈克生物股份有限公司. The sequence listing filed with the application follows.

SEQUENCE LISTING (45 sequences)

SEQ ID NO: 1 - DNA, 59 bp, synthetic construct
  source 1..59: mol_type = other DNA
ccctgggagctcatggaatcgctggtcctgtcgacgctgcgcacactgggacggcaccg

SEQ ID NO: 2 - DNA, 35 bp, synthetic construct
  source 1..35: mol_type = other DNA
cggcaccgaaatattgcagatgtgacaccttagta

SEQ ID NO: 3 - DNA, 37 bp, synthetic construct
  source 1..37: mol_type = other DNA
cgacgctgcgaaatattgcagatgtgacaccttagta

SEQ ID NO: 4 - DNA, 37 bp, synthetic construct
  source 1..37: mol_type = other DNA
ctggtcctgtaaatattgcagatgtgacaccttagta

SEQ ID NO: 5 - DNA, 42 bp, synthetic construct
  source 1..42: mol_type = other DNA
gctcccagggtttaacctggactaagaagaggaacgacagat

SEQ ID NO: 6 - DNA, 35 bp, synthetic construct
  source 1..35: mol_type = other DNA
cgacgctgaaatattgcagatgtgacaccttagta

SEQ ID NO: 7 - DNA, 44 bp, synthetic construct
  source 1..44: mol_type = other DNA
cggtgccgtccctttaacctggactaagaagaggaacgacagat

SEQ ID NO: 8 - DNA, 43 bp, synthetic construct
  source 1..43: mol_type = other DNA
cgacgctgctttggcatcgtattgcagatgtgacaccttagta

SEQ ID NO: 9 - DNA, 51 bp, synthetic construct
  source 1..51: mol_type = other DNA
cggtgccgtcccaaaggcatcgaacctggactaagaagaggaacgacagat

SEQ ID NO: 10 - DNA, 59 bp, synthetic construct
  source 1..59: mol_type = other DNA
tgccaggtcctattgtcacgatcgttagccgtggtccgcacgtcagagcgagtccgagg

SEQ ID NO: 11 - DNA, 59 bp, synthetic construct
  source 1..59: mol_type = other DNA
tcgcaagtgaggcactacgtgagcgatggacggaggcaggagctgtgggaccaggtgcg

SEQ ID NO: 12 - DNA, 59 bp, synthetic construct
  source 1..59: mol_type = other DNA
gactcgagcctcatgaagccgacactgtccgtggagcgactcgaccctgcgacctggca

SEQ ID NO: 13 - DNA, 34 bp, synthetic construct
  source 1..34: mol_type = other DNA
ggacctggcaaaatgcaacatgaccaaggactgg

SEQ ID NO: 14 - DNA, 29 bp, synthetic construct
  source 1..29: mol_type = other DNA
gtccgaggaaatgtagaagccctggtagc

SEQ ID NO: 15 - DNA, 32 bp, synthetic construct
  source 1..32: mol_type = other DNA
ggacctggcaaactaagcagactcacagaact

SEQ ID NO: 16 - DNA, 31 bp, synthetic construct
  source 1..31: mol_type = other DNA
ggtccgcaaaaatgagaacttgccataggtt

SEQ ID NO: 17 - DNA, 35 bp, synthetic construct
  source 1..35: mol_type = other DNA
gcctcacttgcgaaaataactcaaggcggacgatt

SEQ ID NO: 18 - DNA, 30 bp, synthetic construct
  source 1..30: mol_type = other DNA
ccaggtgcgaaattaaccacggcgttcagg

SEQ ID NO: 19 - DNA, 33 bp, synthetic construct
  source 1..33: mol_type = other DNA
gcctcacttgcgaaatggacaacagcagacaac

SEQ ID NO: 20 - DNA, 31 bp, synthetic construct
  source 1..31: mol_type = other DNA
cgatggacaaatccacacgtacaaggtatct

SEQ ID NO: 21 - DNA, 33 bp, synthetic construct
  source 1..33: mol_type = other DNA
ggctcgagtcaaaataatcaggcacgagaacag

SEQ ID NO: 22 - DNA, 32 bp, synthetic construct
  source 1..32: mol_type = other DNA
cgacctggcaaaagactagcaacctccatggc

SEQ ID NO: 23 - DNA, 35 bp, synthetic construct
  source 1..35: mol_type = other DNA
ggctcgagtcaaaaagcaaccaacaacattcattg

SEQ ID NO: 24 - DNA, 32 bp, synthetic construct
  source 1..32: mol_type = other DNA
ccgacactgtaaagcaattcagcatcacagac

SEQ ID NO: 25 - DNA, 20 bp, synthetic construct
  source 1..20: mol_type = other DNA
agcgatggtgtcgagagggt

SEQ ID NO: 26 - DNA, 47 bp, synthetic construct
  source 1..47: mol_type = other DNA
agcgatggtgtcgagagggtaaatattgcagatgtgacaccttagta

SEQ ID NO: 27 - DNA, 29 bp, synthetic construct
  source 1..29: mol_type = other DNA
aacattaagcaagaagaggaaamgaagat

SEQ ID NO: 28 - DNA, 33 bp, synthetic construct
  source 1..33: mol_type = other DNA
ttttttttttactaaggtgtcacatctgcaata

SEQ ID NO: 29 - DNA, 40 bp, synthetic construct
  source 1..40: mol_type = other DNA
cactgggacggcaccgaaaagtctgaacgacctacactcc

SEQ ID NO: 30 - DNA, 16 bp, synthetic construct
  source 1..16: mol_type = other DNA
cccagcagctgacaca

SEQ ID NO: 31 - DNA, 32 bp, synthetic construct
  source 1..32: mol_type = other DNA
gctcatggaaaagtctgaacgacctacactcc

SEQ ID NO: 32 - DNA, 32 bp, synthetic construct
  source 1..32: mol_type = other DNA
gtcgacaggaccatttcccagcagctgacaca

SEQ ID NO: 33 - DNA, 59 bp, synthetic construct
  source 1..59: mol_type = other DNA
gtgcacacggtactgtcagctgaactggtctcactgcagcgctgtccgagctcgacgtg

SEQ ID NO: 34 - DNA, 59 bp, synthetic construct
  source 1..59: mol_type = other DNA
ggcttcgagcacttgcactgatccgatcgacgtgcgaccatgacggagagcaggacgag

SEQ ID NO: 35 - DNA, 34 bp, synthetic construct
  source 1..34: mol_type = other DNA
ccgtgtgcacaaaaaactgacacagggctctgca

SEQ ID NO: 36 - DNA, 35 bp, synthetic construct
  source 1..35: mol_type = other DNA
gctcgacgtgtttgtcatttgccgtgccatacact

SEQ ID NO: 37 - DNA, 36 bp, synthetic construct
  source 1..36: mol_type = other DNA
cgtgtgcacaaatagtagtatggctgcctgatagga

SEQ ID NO: 38 - DNA, 34 bp, synthetic construct
  source 1..34: mol_type = other DNA
tgcagcgctttgtcacccaaataacctagaccgt

SEQ ID NO: 39 - DNA, 32 bp, synthetic construct
  source 1..32: mol_type = other DNA
ccgtgtgcacaaaattggcgaggcacgtatga

SEQ ID NO: 40 - DNA, 38 bp, synthetic construct
  source 1..38: mol_type = other DNA
gctgaactggttttcaccgtcgagccagaaactgtcta

SEQ ID NO: 41 - DNA, 36 bp, synthetic construct
  source 1..36: mol_type = other DNA
gctcgaagccaaaagcaaattggacttcccgtaacg

SEQ ID NO: 42 - DNA, 38 bp, synthetic construct
  source 1..38: mol_type = other DNA
gcgaccatgatttccttctagagaatgcgtgggaatct

SEQ ID NO: 43 - DNA, 59 bp, synthetic construct
  source 1..59: mol_type = other DNA
agacgcacggtgacatgtgtttgactcagttctgctgctgcccaccgtctggagtgcgt

SEQ ID NO: 44 - DNA, 37 bp, synthetic construct
  source 1..37: mol_type = other DNA
ctgctgctgcccaaagcctccttctgcatggtattct

SEQ ID NO: 45 - DNA, 21 bp, synthetic construct
  source 1..21: mol_type = other DNA
agattttgggctggccaaaca